European Patent Application EP 4 215 565 A1, published July 26, 2023. Title: Polyethylene glycol derivatives, composition comprising the same and processes for preparing biological active polypeptide conjugate using the same. Applicant: HANMI PHARM. CO., LTD. HANMI FINE CHEMICAL CO., LTD. The sequence listing filed with the application follows.

SEQUENCE LISTING (4 sequences)

SEQ ID NO: 1 - protein, 34 aa, Artificial Sequence
  Human Glucagon-like peptide-2 derivative
  MISC_FEATURE (1): Xaa is 4-imidazoacetyl (CA)
XGDGSFSDEMNTILDNLAARDFINWLIQTRITDK

SEQ ID NO: 2 - protein, 221 aa, Artificial Sequence
  Human Immunoglobulin Fc fragment
PSCPAPEFLGGPSVFLFPPKPKDTLMISRTPEVTCVVVDVSQEDPEVQFNWYVDGVEVHNAKTKPREEQFNSTYRVVSVLTVLHQDWLNGKEYKCKVSNKGLPSSIEKTISKAKGQPREPQVYTLPPSQEEMTKNQVSLTCLVKGFYPSDIAVEWESNGQPENNYKTTPPVLDSDGSFFLYSRLTVDKSRWQEGNVFSCSVMHEALHNHYTQKSLSLSLGK

SEQ ID NO: 3 - protein, 40 aa, Artificial Sequence
  imidazoacetyl-Exendin-4
  MISC_FEATURE (1): Xaa is 4-imidazoacetyl (CA)
  MISC_FEATURE (40): Xaa is NH2
XGEGTFTSDLSKQMEEEAVRLFIEWLKNGGPSSGAPPPSX

SEQ ID NO: 4 - protein, 174 aa, Artificial Sequence
  granulocyte colony stimulating factor, GCSF
TPLGPASSLPQSFLLKSLEQVRKIQGDGAALQEKLCATYKLCHPEELVLLGHSLGIPWAPLSSCSSQALQLAGCLSQLHSGLFLYQGLLQALEGISPELGPTLDTLQLDVADFATTIWQQMEELGMAPALQPTQGAMPAFASAFQRRAGGVLVASHLQSFLEVSYRVLRHLAQP